European Patent Specification EP 3 828 203 B1, published April 24, 2024. Title: COMPOSITIONS AND METHODS FOR TREATING FATTY TISSUE BUILDUP. Applicant: MHS Care - Innovation LLC. The sequence listing filed with the application follows.

SEQUENCE LISTING (55 sequences)

SEQ ID NO: 1 - protein, 42 aa, Homo sapiens
YAEGTFISDYSIAMDKIHQQDFVNWLLAQKGKKNDWKHNITQ

SEQ ID NO: 2 - protein, 42 aa, Mus musculus
YAEGTFISDYSIAMDKIRQQDFVNWLLAQRGKKSDWKHNITQ

SEQ ID NO: 3 - protein, 42 aa, Rattus norvegicus
YAEGTFISDYSIAMDKIRQQDFVNWLLAQKGKKNDWKHNLTQ

SEQ ID NO: 4 - protein, 42 aa, Sus scrofa
YAEGTFISDYSIAMDKIRQQDFVNWLLAQKGKKSDWKHNITQ

SEQ ID NO: 5 - protein, 18 aa, Artificial Sequence
  artificial screening peptide
YAEGTFISDYSIAMDKIC

SEQ ID NO: 6 - protein, 18 aa, Artificial Sequence
  artificial screening peptide
CLLAQRGKKSDWKHNITQ

SEQ ID NO: 7 - protein, 109 aa, Mus musculus
DIQLTQSPAIMAASLGQKVTMTCSASSSVSSSYLHWYQQKSGASPKSLIHRTSNLASGVPARFSGSGSGTSYSLTISSVEAEDDATYYCLQWSGFPFTFGSGTKLEIKR

SEQ ID NO: 8 - DNA, 327 bp, Artificial Sequence
  artificial
gacattcagctgacccagtctccagcaataatggctgcctctctggggcagaaggtcaccatgacctgcagtgccagctcaagtgtaagttccagttacttgcactggtaccagcagaagtcaggcgcttcccccaaatccttgattcataggacatccaacctggcttctggagtcccagctcgcttcagtggcagtgggtctgggacctcttactctctcacaatcagcagcgtggaggctgaagatgatgcaacttattactgcctgcagtggagtggtttcccattcacgttcggctcggggaccaagctggagatcaaacgt

SEQ ID NO: 9 - protein, 12 aa, Mus musculus
SASSSVSSSYLH

SEQ ID NO: 10 - protein, 9 aa, Mus musculus
LQWSGFPFT

SEQ ID NO: 11 - protein, 117 aa, Mus musculus
QVQLQESGAALVRSGASVKLSCTASGFNIKDYYFHWVKQRPDQGLEWIGWIDPENGDTEYAPNFQVKATMTADTYSNTAYLHLSSLTSEDTAVYYCNSYGNNYFDYWGQGTTVTVSS

SEQ ID NO: 12 - DNA, 351 bp, Artificial Sequence
  artificial
caggtccagctgcaggagtctggggcagcgcttgtgaggtcaggggcctcagtcaaattgtcctgcacagcttctggcttcaacattaaagactactattttcactgggtgaagcagaggcctgaccagggcctggagtggattggatggattgatcctgagaatggtgatactgaatatgccccgaacttccaggtcaaggccactatgactgcagacacatattccaacacagcctacctgcatctcagcagcctgacatctgaggacactgccgtctattactgtaattcctacggtaataactactttgactactggggccaagggaccacggtcaccgtctcctca

SEQ ID NO: 13 - protein, 10 aa, Mus musculus
GFNIKDYYFH

SEQ ID NO: 14 - protein, 7 aa, Mus musculus
APNFQVK

SEQ ID NO: 15 - protein, 10 aa, Mus musculus
NSYGNNYFDY

SEQ ID NO: 16 - protein, 111 aa, Mus musculus
DIQLTQSPSTMAASPGEKITITCSASSSISSNSLHWYQQKPGFSPKLLIYRTSNLASGVPGRFSGSGSGTSYSLTIGTMETEDVATYYCQQGSSFPRMLTFGTGTKLEIKR

SEQ ID NO: 17 - protein, 111 aa, Artificial Sequence
  humanized
DIQMTQSPSSVSASVGDRVTITCRASSSISSNSLHWYQQKPGKAPKLLIYRTSSLQSGVPSRFSGSGSGTDYTLTISSLQPEDFATYYCQQGSSFPRMLTFGQGTKLEIKR

SEQ ID NO: 18 - protein, 111 aa, Artificial Sequence
  humanized
DIQLTQSPSSVSASVGDRVTITCRASSSISSNSLHWYQQKPGKAPKLLIYRTSNLQSGVPSRFSGSGSGTDYTLTISSLQPEDFATYYCQQGSSFPRMLTFGQGTKLEIKR

SEQ ID NO: 19 - protein, 111 aa, Artificial Sequence
  humanized
DIQMTQSPGTLSLSPGERATLSCRASSSISSNSLHWYQQKPGQAPRLLIYRTSNRATGIPARFSGSGSGTDYTLTISSLEPEDFAVYYCQQGSSFPRMLTFGGGTKVEIKR

SEQ ID NO: 20 - protein, 12 aa, Artificial Sequence
  humanized
RASSSISSNSLH

SEQ ID NO: 21 - protein, 7 aa, Artificial Sequence
  humanized
RTSNLQS

SEQ ID NO: 22 - protein, 11 aa, Artificial Sequence
  HUMANIZED
QQGSSFPRMLT

SEQ ID NO: 23 - protein, 7 aa, Artificial Sequence
  HUMANIZED
RTSSLQS

SEQ ID NO: 24 - protein, 7 aa, Artificial Sequence
  HUMANIZED
RTSNRAT

SEQ ID NO: 25 - protein, 12 aa, Artificial Sequence
  HUMANIZED
SASSSISSNSLH

SEQ ID NO: 26 - protein, 7 aa, Mus musculus
RTSNLAS

SEQ ID NO: 27 - protein, 117 aa, Mus musculus
QVQLQESGAELVRSGASVKLSCTASGFNIRDYYLHWIKQRPEQGLEWIGWIDPENGDTEYAPKFQDKATVTADTSSNTAYLQLNSLTSEDTAVYYCNVYGIYFMDYWGQGTTVTVSS

SEQ ID NO: 28 - protein, 117 aa, Artificial Sequence
  HUMANIZED
QVQLVQSGAEVKKPGATVKISCKVSGFNIRDYYLHWVQQAPGKGLEWMGWIDPENGDTEYAPKFQGRVTITADTSTDTAYMELSSLRSEDTAVYYCNVYGIYFMDYWGQGTMVTVSS

SEQ ID NO: 29 - protein, 117 aa, Artificial Sequence
  HUMANIZED
QVQLVQSGAEVKKPGATVKISCKASGFNIRDYYLHWVQQAPGKGLEWMGWIDPENGDTEYAPKFQGRVTITADTSTNTAYMELSSLRSEDTAVYYCNVYGIYFMDYWGQGTMVTVSS

SEQ ID NO: 30 - protein, 117 aa, Artificial Sequence
  HUMANIZED
QVQLQESGAEVKKPGASVKVSCKASGFNIRDYYLHWVRQAPGQGLEWMGWIDPENGDTEYAPKFQGRVTTTADTSISTAYMELSRLRSDDTAVYYCNVYGIYFMDYWGQGTLVTVSS

SEQ ID NO: 31 - protein, 10 aa, Mus musculus
GFNIRDYYLH

SEQ ID NO: 32 - protein, 7 aa, Artificial Sequence
  HUMANIZED
APKFQGR

SEQ ID NO: 33 - protein, 10 aa, Mus musculus
NVYGIYFMDY

SEQ ID NO: 34 - protein, 7 aa, Mus musculus
APKFQDK

SEQ ID NO: 35 - DNA, 333 bp, Artificial Sequence
  ARTIFICIAL
gacattcagctgacccagtctccatccaccatggctgcatctcccggggagaagatcactatcacctgcagtgccagctcaagtataagttccaattccttgcattggtatcagcagaagccaggattctcccctaaactcttgatttataggacatccaatctggcttctggagtcccaggtcgcttcagtggcagtgggtctgggacctcttactctctcacaattggcaccatggagactgaagatgttgccacttactactgccagcagggtagtagttttccacgcatgctcacgttcggtactgggaccaagctggagatcaaacgt

SEQ ID NO: 36 - DNA, 333 bp, Artificial Sequence
  ARTIFICIAL
gacatccagatgacccagtccccctcctccgtgtctgcttctgtgggcgacagagtgacaattacctgccgggcctcctcctccatctcctccaattccctgcactggtatcagcagaagcccggcaaggcccccaagctgctgatctaccggacctccagcctgcagtccggcgtgccctctagattctccggctctggctctggcaccgactataccctgaccatctccagcctgcagcccgaggacttcgccacctactactgtcagcagggctcctccttcccccggatgctgacatttggccagggcaccaagctggaaatcaagcgg

SEQ ID NO: 37 - DNA, 333 bp, Artificial Sequence
  ARTIFICIAL
gacatccagctgacccagtccccctcctccgtgtctgcttctgtgggcgacagagtgacaattacctgccgggcctcctcctccatctcctccaattccctgcactggtatcagcagaagcccggcaaggcccccaagctgctgatctaccggacctccaacctgcagtccggcgtgccctctagattctccggctctggctctggcaccgactataccctgaccatctccagcctgcagcccgaggacttcgccacctactactgtcagcagggctcctccttcccccggatgctgacatttggccagggcaccaagctggaaatcaagcgg

SEQ ID NO: 38 - DNA, 333 bp, Artificial Sequence
  ARTIFICIAL
gacatccagatgacccagagccctggcaccctgtctctgtctcccggcgagagagctaccctgtcctgcagagcctcctcctccatctcctccaattccctgcactggtatcagcagaagcccggccaggcccccagactgctgatctaccggacctccaatcgggccaccggcatccctgccagattctccggctctggctctggcaccgactataccctgaccatctccagcctggaacccgaggacttcgccgtgtactactgtcagcagggctcctccttcccccggatgctgacatttggcggaggcaccaaggtggaaatcaagcgg

SEQ ID NO: 39 - DNA, 351 bp, Artificial Sequence
  ARTIFICIAL
caggtccagctgcaggagtctggggcagagcttgtgaggtcaggggcctcagtcaagttgtcctgcacagcttctggcttcaacattagagactactatttgcactggataaaacagaggcctgaacagggcctggagtggattggatggattgatcctgagaatggtgatactgaatatgccccgaagttccaggacaaggccactgtgactgcagacacatcctccaacacagcctacctgcagctcaacagcctgacatctgaggacactgccgtctattactgtaatgtatatggcatctattttatggactattggggccaagggaccacggtcaccgtctcctca

SEQ ID NO: 40 - DNA, 351 bp, Artificial Sequence
  ARTIFICIAL
caggtgcagctggtgcagtctggcgccgaagtgaagaaacctggcgctaccgtgaagatctcctgcaaggtgtccggcttcaacatccgggactactacctgcactgggtgcagcaggcccctggcaagggactggaatggatgggctggatcgaccccgagaacggcgataccgagtacgcccctaagttccagggcagagtgaccatcaccgccgacacctctaccgacaccgcctacatggaactgtcctccctgcggagcgaggacaccgccgtgtactactgcaacgtgtacggcatctacttcatggactactggggccagggcacaatggtcaccgtgtcctct

SEQ ID NO: 41 - DNA, 351 bp, Artificial Sequence
  ARTIFICIAL
caggtgcagctggtgcagtctggcgccgaagtgaagaaacctggcgctaccgtgaagatctcctgcaaggcctccggcttcaacatccgggactactacctgcactgggtgcagcaggcccctggcaagggactggaatggatgggctggatcgaccccgagaacggcgataccgagtacgcccctaagttccagggcagagtgaccatcaccgccgacacctctaccaacaccgcctacatggaactgtcctccctgcggagcgaggacaccgccgtgtactactgcaacgtgtacggcatctacttcatggactactggggccagggcacaatggtcaccgtgtcctct

SEQ ID NO: 42 - DNA, 351 bp, Artificial Sequence
  artificial
caggtgcagctgcaggaatctggcgccgaagtgaagaaacctggcgcctccgtgaaggtgtcctgcaaggcctccggcttcaacatccgggactactacctgcactgggtgcgacaggctccaggccagggactggaatggatgggctggatcgaccccgagaacggcgataccgagtacgcccctaagttccagggcagagtgaccaccaccgccgacacctctatctccaccgcctacatggaactgtcccggctgagatccgacgacaccgccgtgtactactgcaacgtgtacggcatctacttcatggactactggggccagggcacactcgtcaccgtgtcctct

SEQ ID NO: 43 - protein, 46 aa, Artificial Sequence
  primer
CAGTCGAAGCTTTGAGGAGACGGTGACCGTGGTCCCTTGGCCCCAG

SEQ ID NO: 44 - protein, 34 aa, Artificial Sequence
  primer
CAACTAGGATCCAGGTSMARCTGCAGSAGTCWGG

SEQ ID NO: 45 - protein, 6 aa, Artificial Sequence
  primer
AAGCTT

SEQ ID NO: 46 - protein, 6 aa, Artificial Sequence
  primer
GGATCC

SEQ ID NO: 47 - protein, 34 aa, Artificial Sequence
  primer
CAGTCGAAGCTTGTTAGATCTCCAGCTTGGTCCC

SEQ ID NO: 48 - DNA, 36 bp, Artificial Sequence
  primer
caactaggatccgacattcagctgacccagtctcca

SEQ ID NO: 49 - DNA, 30 bp, Artificial Sequence
  primer
tcacgaattctcaggtccagctgcaggagt

SEQ ID NO: 50 - DNA, 29 bp, Artificial Sequence
  primer
ttggtgctagctgaggagacggtgaccgt

SEQ ID NO: 51 - DNA, 6 bp, Artificial Sequence
  primer
gaattc

SEQ ID NO: 52 - DNA, 6 bp, Artificial Sequence
  primer
gctagc

SEQ ID NO: 53 - DNA, 34 bp, Artificial Sequence
  primer
agccaccgtacgtttgatctccagcttggtccca

SEQ ID NO: 54 - DNA, 6 bp, Artificial Sequence
  primer
cgtacg

SEQ ID NO: 55 - protein, 30 aa, Artificial Sequence
  primer
GTCACGAATTCAGACATTCAGCTGACCCAG